European Patent Specification EP 3 565 902 B1, published September 4, 2024. Title: Procédé de détection et quantification d'ADN circulant et utilisations. Applicant: cfID.Solutions. The sequence listing filed with the application follows.

SEQUENCE LISTING (11 sequences)

SEQ ID NO: 1 - DNA, 300 bp, artificial
  1er fragment d'ADN exogène 300pb codant pour le précurseur d une protéase à  serine pro-agrégante de Cerastes cerastes
cctaatgacacttatcccaaagtccctcattgtgctaacattaacatacttgagcattcgctgtgtgaaagagcttacaatgatctttcggcgagtagcagaacattgtgtgcaggtatcgaaaaaggaggcatagatacatgtaagggtgactctgggggacccctcatctgtaatggacaaatccagggcattgtatcttggggagatgaagtttgtggtaaacctaataagcctggcgtctataccaaggtctttgattatactgactggatccggaacattattgcaggaaataca

SEQ ID NO: 2 - DNA, 110 bp, artificial
  2nd fragment d'ADN exogène 110pb codant pour le précurseur d une protéase à  serine pro-agrégante de Cerastes cerastes
gctgaacaaaccagttaacaacagtacacacatcgcgcctctcagcttgccttccagtcctcccagtgtgggctcagattgccgtattatgggatggggcacaatcacat

SEQ ID NO: 3 - DNA, 22 bp, artificial
  amorce sens dirigée contre 1er fragment
tggacaaggacatcatgctgat

SEQ ID NO: 4 - DNA, 20 bp, artificial
  amorce antisens dirigée contre  1er fragment
gactggaaggcaagctgaga

SEQ ID NO: 5 - DNA, 30 bp, artificial
  sonde marquée dirigée contre  1er fragment
aaccagttaacaacagtacacacatcgcgc

SEQ ID NO: 6 - DNA, 18 bp, artificial
  amorce sens dirigée contre  gène RPP-30 humain
gatttggacctgcgagcg

SEQ ID NO: 7 - DNA, 20 bp, artificial
  amorce antisens dirigée contre  gène RPP-30 humain
gagcggctgtctccacaagt

SEQ ID NO: 8 - DNA, 16 bp, artificial
  sonde marquée dirigée contre gène RPP-30 humain
ctgacctgaaggctct

SEQ ID NO: 9 - DNA, 24 bp, artificial
  amorce sens dirigée contre 2nd fragment
atgacacttatcccaaagtccctc

SEQ ID NO: 10 - DNA, 21 bp, artificial
  amorce antisens dirigée contre  2nd fragment
caatgttctgctactcgccga

SEQ ID NO: 11 - DNA, 20 bp, artificial
  sonde marquée dirigée contre  2nd fragment
catacttgagcattcgctgt